European Patent Application EP 4 154 867 A1, published March 29, 2023. Title: A liquid formulation. Applicant: HANMI PHARM. CO., LTD. The sequence listing filed with the application follows.

SEQUENCE LISTING (26 sequences)

SEQ ID NO: 1 - protein, 30 aa, Artificial Sequence
  Formula 1 of oxyntomodulin derivative
  VARIANT (2): Xaa = 2-aminoisobutyric acid
  VARIANT (12): Xaa = Lysine
  VARIANT (16): Xaa = glutamic acid
  VARIANT (20): Xaa = Lysine
HXQGTFTSDYSXYLDXKRAXEFVQWLMNTC

SEQ ID NO: 2 - protein, 30 aa, Artificial Sequence
  oxyntomodulin derivative
  VARIANT (2): Xaa = 2-aminoisobutyric acid
HXQGTFTSDYSKYLDEKRAKEFVQWLMNTC

SEQ ID NO: 3 - protein, 30 aa, Artificial Sequence; identical to SEQ ID NO: 2
  oxyntomodulin derivative
  VARIANT (2): Xaa = 2-aminoisobutyric acid
  VARIANT (16)..(20): amino acids at position 16 and position 20 form a ring

SEQ ID NO: 4 - protein, 30 aa, Artificial Sequence; identical to SEQ ID NO: 2
  oxyntomodulin derivative
  VARIANT (2): Xaa = 2-aminoisobutyric acid
  VARIANT (12)..(16): amino acids at position 12 and position 16 form a ring

SEQ ID NO: 5 - protein, 221 aa, homo sapiens
PSCPAPEFLGGPSVFLFPPKPKDTLMISRTPEVTCVVVDVSQEDPEVQFNWYVDGVEVHNAKTKPREEQFNSTYRVVSVLTVLHQDWLNGKEYKCKVSNKGLPSSIEKTISKAKGQPREPQVYTLPPSQEEMTKNQVSLTCLVKGFYPSDIAVEWESNGQPENNYKTTPPVLDSDGSFFLYSRLTVDKSRWQEGNVFSCSVMHEALHNHYTQKSLSLSLGK

SEQ ID NO: 6 - protein, 12 aa, homo sapiens
ESKYGPPCPSCP

SEQ ID NO: 7 - protein, 11 aa, Artificial Sequence
  Variant of hinge region
ESKYGPPPSCP

SEQ ID NO: 8 - protein, 11 aa, Artificial Sequence
  Variant of hinge region
ESKYGPPCPSP

SEQ ID NO: 9 - protein, 10 aa, Artificial Sequence
  Variant of hinge region
ESKYGPPCPS

SEQ ID NO: 10 - protein, 10 aa, Artificial Sequence
  Variant of hinge region
ESKYGPPCPP

SEQ ID NO: 11 - protein, 8 aa, Artificial Sequence
  Variant of hinge region
KYGPPCPS

SEQ ID NO: 12 - protein, 8 aa, Artificial Sequence
  Variant of hinge region
ESKYGPPC

SEQ ID NO: 13 - protein, 7 aa, Artificial Sequence
  Variant of hinge region
EKYGPPC

SEQ ID NO: 14 - protein, 6 aa, Artificial Sequence
  Variant of hinge region
ESPSCP

SEQ ID NO: 15 - protein, 5 aa, Artificial Sequence
  Variant of hinge region
EPSCP

SEQ ID NO: 16 - protein, 4 aa, Artificial Sequence
  Variant of hinge region
PSCP

SEQ ID NO: 17 - protein, 10 aa, Artificial Sequence
  Variant of hinge region
ESKYGPPSCP

SEQ ID NO: 18 - protein, 9 aa, Artificial Sequence
  Variant of hinge region
KYGPPPSCP

SEQ ID NO: 19 - protein, 9 aa, Artificial Sequence
  Variant of hinge region
ESKYGPSCP

SEQ ID NO: 20 - protein, 8 aa, Artificial Sequence
  Variant of hinge region
ESKYGPPC

SEQ ID NO: 21 - protein, 7 aa, Artificial Sequence
  Variant of hinge region
KYGPPCP

SEQ ID NO: 22 - protein, 7 aa, Artificial Sequence
  Variant of hinge region
ESKPSCP

SEQ ID NO: 23 - protein, 6 aa, Artificial Sequence
  Variant of hinge region
ESPSCP

SEQ ID NO: 24 - protein, 4 aa, Artificial Sequence
  Variant of hinge region
EPSC

SEQ ID NO: 25 - protein, 3 aa, Artificial Sequence
  Variant of hinge region
SCP

SEQ ID NO: 26 - protein, 442 aa, Homo sapiens
  MISC_FEATURE (1)..(442): Amino acids at position 1 to 442 form Human Immunoglobulin G4 Fc Fragment (homodimer)
  MISC_FEATURE (1)..(221): Amino acids at position 1 to 221 form one monomer
  MISC_FEATURE (222)..(442): Amino acids at position 222 to 442 form one monomer
  DISULFID (3)..(224): Amino acids at position 3 and position 224 form an inter-disulfide bond
  DISULFID (35)..(95): Amino acids at position 35 and position 95 form an intra-chain disulfide bond
  DISULFID (141)..(199): Amino acids at position 141 and position 199 form an intra-chain disulfide bond
  DISULFID (256)..(316): Amino acids at position 256 and position 316 form an intra-chain disulfide bond
  DISULFID (362)..(420): Amino acids at position 362 and position 420 form an intra-chain disulfide bond
PSCPAPEFLGGPSVFLFPPKPKDTLMISRTPEVTCVVVDVSQEDPEVQFNWYVDGVEVHNAKTKPREEQFNSTYRVVSVLTVLHQDWLNGKEYKCKVSNKGLPSSIEKTISKAKGQPREPQVYTLPPSQEEMTKNQVSLTCLVKGFYPSDIAVEWESNGQPENNYKTTPPVLDSDGSFFLYSRLTVDKSRWQEGNVFSCSVMHEALHNHYTQKSLSLSLGKPSCPAPEFLGGPSVFLFPPKPKDTLMISRTPEVTCVVVDVSQEDPEVQFNWYVDGVEVHNAKTKPREEQFNSTYRVVSVLTVLHQDWLNGKEYKCKVSNKGLPSSIEKTISKAKGQPREPQVYTLPPSQEEMTKNQVSLTCLVKGFYPSDIAVEWESNGQPENNYKTTPPVLDSDGSFFLYSRLTVDKSRWQEGNVFSCSVMHEALHNHYTQKSLSLSLGK